European Patent Specification EP 3 079 718 B1, published April 9, 2025. Title: HUMAN HERPESVIRUS TRIMERIC GLYCOPROTEIN B VACCINE. Applicant: THE HENRY M. JACKSON FOUNDATION FOR THE ADVANCEMENT OF MILITARY MEDICINE, INC. The sequence listing filed with the application follows.

SEQUENCE LISTING (26 sequences)

SEQ ID NO: 1 - DNA, 2724 bp, Human cytomegalovirus
tcagacgttctcttcttcgtcagagtctttcaagtgtcggtagccgtttttgcgatgtcgcagtcggtctagtaggttgggcttctgtcccttgtcctgcgtgccagtccgtccgtccaaagaatctgtaccgttctgctgcgctcgctgctctgcgtccagacgggccagggccagaagcatctggtaagcctgctcgttggtgtaaggcggagccgccgtggatgcatcagacgacggtggtcccggtcctttgcgaccagaattataaacactttcctcgtaggaaggcggagcctgtaacgacgtgtctttggtgctgcccgacgtcacggtggtcccgtcggcggacaccagatagggaaagaggttctgcagcggctgcgtgcacaaacgccgctgtcgagtatagatcaaataagtgataatgactacagctatggccacgaggatgatggtgaacgctccgaaggggtttttgaggaaggtggcaacgccttcgaccacggaggccaccgcgccacccacggccccaatggctacgccaacggcctttcccgcggcgcccaggccgctcatgaggtcgtccagacccttgaggtagggcggtagcgggtcgactaccttgtcctccacgtactttacccgctgcttgtacgagttgaattcgcgcatgatctcttcgaggtcaaaaacgttgctggaacgcagctctttctgcgagtaaagttccagtaccctgaagtcggtattttccagcgggtcgatatccagggcgatcatgctgtcgacggtggagatactgctgaggtcaatcatgcgtttgaagaggtagtccacgtactcgtaggccgagttcccggcgatgaagatcttgaggctgggaagctgacattcctcagtgcggtggttgcccaacaggatttcgttgtcctcgcccagttgaccgtactgcacgtacgagctgttggcgaaattaaagatgaccacgggtcgtgagtagcagcgtcctggcgactccttcacgttcatatcacgcagcaccttgacgctggtttggttgatggtcacgcagctggccaggcccaagacatcacccatgaaacgcgcggcaatcggtttgttgtaaatggccgagagaatggctgacgggttgatcttgctgagttccttgaagacctctagggtgcgccgttgatccacacaccaggcttctgcgatttgcgccagcgcccggttgatgtaaccgcgcaacgtgtcataggtgaactgcagctgggcgtagaccagattgtgcaccgattccatgttggataaatgagttgcattgttgccatctgtacttcttttggttctattatgagtaagattcagactggagcggttggccaaacgttcgagttccaccagagatttttgcttgataccttgccagaacactaccaaaccaccagtggtttcaaagacggacacgtttccatatttttcatatgtttgattgtatgaagtattgaaaatctgctgtaacttatttatagcctcatcacgtacgcagtccagcgcagagtcggacatgttcacctcttgcttcttagataagaaagtggcggtcattttggcagaagaaaagtgatacgagtcctcggcttcggaacgaatggtgcgttccgaggcttcccagaaagtgagttgacaagtgacattcttttcgtcctgtatatcccaggagatcaccgagtccgcacgttcaagaaaagccaccaacctgtgggtctctaacgcagaattcggtcttccaaagtcggagacgatagtgtagttcggaaaaatgaaaaacttgtcggcgttttctccaaagtagctggcattgcgattggttccgttgtagaaaggagaaatgtcaaccacgtcacccgtggaagtggcgaaaaaatgataaggatatttggagcgcgcagtagtgatggtcaccatacaattcagattacaggtctcacgatagagccaggtgctgccgcggctgtgccattgatccttgaccgtcacgtaacgggtactgtgggtgttggaataatcgtcgggcattaattgcatggttttgttttcatagctgtccctatgataagccacgaaaaccgtgcctgctataacgcggctgtaggaactgtagcactgactgtggctgttgatatgatgaatctcccacataggaggcgccacgtattccgtgttgctgcccagcagataagtggtgtggatgtaagcgtagctacgacgaaacgtcaaaaccttctggtagactcgtaccttaaaggtgtgcgcgacgatgttgcgtttgtagaccaccatgatgccctcgtccaggtcttcattgatgggcttcatcgaggtgcagacgatattacgttcaaagcgaataagatccgtaccctgggccatagaacacacgcgataggggtacttggtggtattgacccccaccacatctccgtacttgagggtagtgttgtagatggtctcgttaacaccatggctgaccgtttgggaagaagttacgcgttgagagactgaaccggatcgagagtgagcagcagacgtcgtatgagaggaatggtgactgtgagtagcagaagttccacgagtagaagatgaggaaaccgcagcacccagacagacgatacacaagttaacgcagactaccaggcaccagatcctggattccat

SEQ ID NO: 2 - protein, 907 aa, Human cytomegalovirus
MESRIWCLVVCVNLCIVCLGAAVSSSSTRGTSATHSHHSSHTTSAAHSRSGSVSQRVTSSQTVSHGVNETIYNTTLKYGDVVGVNTTKYPYRVCSMAQGTDLIRFERNIVCTSMKPINEDLDEGIMVVYKRNIVAHTFKVRVYQKVLTFRRSYAYIHTTYLLGSNTEYVAPPMWEIHHINSHSQCYSSYSRVIAGTVFVAYHRDSYENKTMQLMPDDYSNTHSTRYVTVKDQWHSRGSTWLYRETCNLNCMVTITTARSKYPYHFFATSTGDVVDISPFYNGTNRNASYFGENADKFFIFPNYTIVSDFGRPNSALETHRLVAFLERADSVISWDIQDEKNVTCQLTFWEASERTIRSEAEDSYHFSSAKMTATFLSKKQEVNMSDSALDCVRDEAINKLQQIFNTSYNQTYEKYGNVSVFETTGGLVVFWQGIKQKSLVELERLANRSSLNLTHNRTKRSTDGNNATHLSNMESVHNLVYAQLQFTYDTLRGYINRALAQIAEAWCVDQRRTLEVFKELSKINPSAILSAIYNKPIAARFMGDVLGLASCVTINQTSVKVLRDMNVKESPGRCYSRPVVIFNFANSSYVQYGQLGEDNEILLGNHRTEECQLPSLKIFIAGNSAYEYVDYLFKRMIDLSSISTVDSMIALDIDPLENTDFRVLELYSQKELRSSNVFDLEEIMREFNSYKQRVKYVEDKVVDPLPPYLKGLDDLMSGLGAAGKAVGVAIGAVGGAVASVVEGVATFLKNPFGAFTIILVAIAVVIITYLIYTRQRRLCTQPLQNLFPYLVSADGTTVTSGSTKDTSLQAPPSYEESVYNSGRKGPGPPSSDASTAAPPYTNEQAYQMLLALARLDAEQRAQQNGTDSLDGRTGTQDKGQKPNLLDRLRHRKNGYRHLKDSDEEENV

SEQ ID NO: 3 - DNA, 2343 bp, Artificial Sequence
  Description of Artificial Sequence: Synthetic polynucleotide
atggagacagacacactcctgctatgggtactgctgctctgggttccaggttccactggtgacgcggcccagccggccaggcgcgcgcgccgtacgaagctcgcccttgtttcctcatcttctactcgtggaacttctgctactcacagtcaccattcctctcatacgacgtctgctgctcactctcgatccggttcagtctctcaacgcgtaacttcttcccaaacggtcagccatggtgttaacgagaccatctacaacactaccctcaagtacggagatgtggtgggggtcaataccaccaagtacccctatcgcgtgtgttctatggcccagggtacggatcttattcgctttgaacgtaatatcgtctgcacctcgatgaagcccatcaatgaagacctggacgagggcatcatggtggtctacaaacgcaacatcgtcgcgcacacctttaaggtacgagtctaccagaaggttttgacgtttcgtcgtagctacgcttacatccacaccacttatctgctgggcagcaacacggaatacgtggcgcctcctatgtgggagattcatcatatcaacagccacagtcagtgctacagttcctacagccgcgttatagcaggcacggttttcgtggcttatcatagggacagctatgaaaacaaaaccatgcaattaatgcccgacgattattccaacacccacagtacccgttacgtgacggtcaaggatcaatggcacagccgcggcagcacctggctctatcgtgagacctgtaatctgaattgtatggtgaccatcactactgcgcgctccaaatatccttatcattttttcgccacttccacgggtgacgtggttgacatttctcctttctacaacggaaccaatcgcaatgccagctactttggagaaaacgccgacaagtttttcatttttccgaactacactatcgtctccgactttggaagaccgaattctgcgttagagacccacaggttggtggcttttcttgaacgtgcggactcggtgatctcctgggatatacaggacgaaaagaatgtcacttgtcaactcactttctgggaagcctcggaacgcaccattcgttccgaagccgaggactcgtatcacttttcttctgccaaaatgaccgccactttcttatctaagaagcaagaggtgaacatgtccgactctgcgctggactgcgtacgtgatgaggctataaataagttacagcagattttcaatacttcatacaatcaaacatatgaaaaatatggaaacgtgtccgtctttgaaaccactggtggtttggtagtgttctggcaaggtatcaagcaaaaatctctggtggaactcgaacgtttggccaaccgctccagtctgaatcttactcataatggtggcggagggagtggtggcggagggagcggtggcggagggagtacagatggcaacaatgcaactcatttatccaacatggaatcggtgcacaatctggtctacgcccagctgcagttcacctatgacacgttgcgcggttacatcaaccgggcgctggcgcaaatcgcagaagcctggtgtgtggatcaacggcgcaccctagaggtcttcaaggaactcagcaagatcaacccgtcagccattctctcggccatttacaacaaaccgattgccgcgcgtttcatgggtgatgtcttgggcctggccagctgcgtgaccatcaaccaaaccagcgtcaaggtgctgcgtgatatgaacgtgaaggagtcgccaggacgctgctactcacgacccgtggtcatctttaatttcgccaacagctcgtacgtgcagtacggtcaactgggcgaggacaacgaaatcctgttgggcaaccaccgcactgaggaatgtcagcttcccagcctcaagatcttcatcgccgggaactcggcctacgagtacgtggactacctcttcaaacgcatgattgacctcagcagtatctccaccgtcgacagcatgatcgccctggatatcgacccgctggaaaataccgacttcagggtactggaactttactcgcagaaagagctgcgttccagcaacgtttttgacctcgaagagatcatgcgcgaattcaactcgtacaagcagcgggtaaagtacgtggaggacaaggtagtcgacccgctaccgccctacctcaagggtctggacgacctcatgagcggcctgggcgccgcgggaaaggccgttggcgtagccattggggccgtgggtggcgcggtggcctccgtggtcgaaggcgttgccaccttcctcaaaaaccatcatcaccatcaccattga

SEQ ID NO: 4 - protein, 780 aa, Artificial Sequence
  Description of Artificial Sequence: Synthetic polypeptide
METDTLLLWVLLLWVPGSTGDAAQPARRARRTKLALVSSSSTRGTSATHSHHSSHTTSAAHSRSGSVSQRVTSSQTVSHGVNETIYNTTLKYGDVVGVNTTKYPYRVCSMAQGTDLIRFERNIVCTSMKPINEDLDEGIMVVYKRNIVAHTFKVRVYQKVLTFRRSYAYIHTTYLLGSNTEYVAPPMWEIHHINSHSQCYSSYSRVIAGTVFVAYHRDSYENKTMQLMPDDYSNTHSTRYVTVKDQWHSRGSTWLYRETCNLNCMVTITTARSKYPYHFFATSTGDVVDISPFYNGTNRNASYFGENADKFFIFPNYTIVSDFGRPNSALETHRLVAFLERADSVISWDIQDEKNVTCQLTFWEASERTIRSEAEDSYHFSSAKMTATFLSKKQEVNMSDSALDCVRDEAINKLQQIFNTSYNQTYEKYGNVSVFETTGGLVVFWQGIKQKSLVELERLANRSSLNLTHNGGGGSGGGGSGGGGSTDGNNATHLSNMESVHNLVYAQLQFTYDTLRGYINRALAQIAEAWCVDQRRTLEVFKELSKINPSAILSAIYNKPIAARFMGDVLGLASCVTINQTSVKVLRDMNVKESPGRCYSRPVVIFNFANSSYVQYGQLGEDNEILLGNHRTEECQLPSLKIFIAGNSAYEYVDYLFKRMIDLSSISTVDSMIALDIDPLENTDFRVLELYSQKELRSSNVFDLEEIMREFNSYKQRVKYVEDKVVDPLPPYLKGLDDLMSGLGAAGKAVGVAIGAVGGAVASVVEGVATFLKNHHHHHH

SEQ ID NO: 5 - protein, 15 aa, Artificial Sequence
  Description of Artificial Sequence: Synthetic peptide
GGGGSGGGGSGGGGS

SEQ ID NO: 6 - protein, 21 aa, Artificial Sequence
  Description of Artificial Sequence: Synthetic peptide
METDTLLLWVLLLWVPGSTGD

SEQ ID NO: 7 - DNA, 2574 bp, Epstein-Barr virus
atgactcggcgtagggtgctaagcgtggtcgtgctgctagccgccctggcgtgccgcctcggtgcgcagaccccagagcagcccgcaccccccgccaccacggtgcagcctaccgccacgcgtcagcaaaccagctttcctttccgagtctgcgagctctccagccacggcgacctgttccgcttctcctcggacatccagtgtccctcgtttggcacgcgggagaatcacacggagggcctgttgatggtgtttaaagacaacattattccctactcgtttaaggtccgctcctacaccaagatagtgaccaacattctcatctacaatggctggtacgcggactccgtgaccaaccggcacgaggagaagttctccgttgacagctacgaaactgaccagatggataccatctaccagtgctacaacgcggtcaagatgacaaaagatgggctgacgcgcgtgtatgtagaccgcgacggagttaacatcaccgtcaacctaaagcccaccgggggcctggccaacggggtgcgccgctacgccagccagacggagctctatgacgcccccgggtggttgatatggacttacagaacaagaactaccgtcaactgcctgataactgacatgatggccaagtccaacagccccttcgacttctttgtgaccaccaccgggcagactgtggaaatgtcccctttctatgacgggaaaaataaggaaaccttccatgagcgggcagactccttccacgtgagaactaactacaagatagtggactacgacaaccgagggacgaacccgcaaggcgaacgccgagccttcctggacaagggcacttacaccctatcttggaagctcgagaacaggacagcctactgcccgcttcaacactggcaaacctttgactcgaccatcgccacagaaacagggaagtcaatacattttgtgactgacgagggcacctctagcttcgtgaccaacacaaccgtgggcatagagctcccggacgccttcaagtgcatcgaagagcaggtgaacaagaccatgcatgagaagtacgaggccgtccaggatcgttacacgaagggccaggaagccattacatattttataacgagcggaggattgttattagcttggctacctctgaccccgcgctcgttggccaccgtcaagaacctgacggagcttaccactccgacttcctcaccccccagcagtccatcgccccccgccccacccgcggcccgcgggagcacctccgccgccgttctgaggcgccggaggcgggatgcggggaatgccaccacaccggtgccccccgcggcccccgggaagtccctgggcaccctcaacaatcccgccaccgtccagatccaatttgcctacgattccctgcgccgccagatcaaccgcatgctgggagacctcgcgcgggcctggtgcctggagcagaagaggcagaacatggtgctgagagaactaaccaagattaatcccaccaccgtcatgtccagcatctacggtaaggcggtggcggccaagcgcctgggggatgtcatctcagtctcccagtgcgtgcccgttaaccaggccaccgtcaccctgcgcaagagcatgagggtccctggctccgagaccatgtgctactcgcgccccctggtgtccttcagctttatcaacgacaccaagacctacgagggacagctgggcaccgacaacgagatcttcctcacaaaaaagatgacggaggtgtgccaggcgaccagccagtactacttccagtccggcaacgagatccacgtctacaacgactaccaccactttaaaaccatcgagctggacggcattgccaccctgcagaccttcatctcactaaacacctccctcatcgagaacattgactttgcctccctggagctgtactcacgggacgaacagcgtgcctccaacgtctttgacctggagggcatcttccgggagtacaacttccaggcgcaaaacatcgccggcctgcggaaggatttggacaatgcagtgtcaaacggaagaaatcaattcgtggacggcctgggggaacttatggacagtctgggtagcgtgggtcagtccatcaccaacctagtcagcacggtggggggtttgtttagcagcctggtctctggtttcatctccttcttcaaaaaccccttcggcggcatgctcattctggtcctggtggcgggggtggtgatcctggttatttccctcacgaggcgcacgcgccagatgtcgcagcagccggtgcagatgctctaccccgggatcgacgagctcgctcagcaacatgcctctggtgagggtccaggcattaatcccattagtaagacagaattacaagccatcatgttagcgctgcatgagcaaaaccaggagcaaaagagagcagctcagagggcggccggaccctcagtggccagcagagcattgcaggcagccagggaccgttttccaggcctacgcagaagacgctatcacgatccagagaccgccgccgcactgcttggggaggcagagactgagttttaa

SEQ ID NO: 8 - protein, 857 aa, Epstein-Barr virus
MTRRRVLSVVVLLAALACRLGAQTPEQPAPPATTVQPTATRQQTSFPFRVCELSSHGDLFRFSSDIQCPSFGTRENHTEGLLMVFKDNIIPYSFKVRSYTKIVTNILIYNGWYADSVTNRHEEKFSVDSYETDQMDTIYQCYNAVKMTKDGLTRVYVDRDGVNITVNLKPTGGLANGVRRYASQTELYDAPGWLIWTYRTRTTVNCLITDMMAKSNSPFDFFVTTTGQTVEMSPFYDGKNKETFHERADSFHVRTNYKIVDYDNRGTNPQGERRAFLDKGTYTLSWKLENRTAYCPLQHWQTFDSTIATETGKSIHFVTDEGTSSFVTNTTVGIELPDAFKCIEEQVNKTMHEKYEAVQDRYTKGQEAITYFITSGGLLLAWLPLTPRSLATVKNLTELTTPTSSPPSSPSPPAPPAARGSTSAAVLRRRRRDAGNATTPVPPAAPGKSLGTLNNPATVQIQFAYDSLRRQINRMLGDLARAWCLEQKRQNMVLRELTKINPTTVMSSIYGKAVAAKRLGDVISVSQCVPVNQATVTLRKSMRVPGSETMCYSRPLVSFSFINDTKTYEGQLGTDNEIFLTKKMTEVCQATSQYYFQSGNEIHVYNDYHHFKTIELDGIATLQTFISLNTSLIENIDFASLELYSRDEQRASNVFDLEGIFREYNFQAQNIAGLRKDLDNAVSNGRNQFVDGLGELMDSLGSVGQSITNLVSTVGGLFSSLVSGFISFFKNPFGGMLILVLVAGVVILVISLTRRTRQMSQQPVQMLYPGIDELAQQHASGEGPGINPISKTELQAIMLALHEQNQEQKRAAQRAAGPSVASRALQAARDRFPGLRRRRYHDPETAAALLGEAETEF

SEQ ID NO: 9 - DNA, 2235 bp, Epstein-Barr virus
atggagacagacacactcctgctatgggtactgctgctctgggttccaggttccactggtgacgcggcccagaccccagagcagcccgcaccccccgccaccacggtgcagcctaccgccacgcgtcagcaaaccagctttcctttccgagtctgcgagctctccagccacggcgacctgttccgcttctcctcggacatccagtgtccctcgtttggcacgcgggagaatcacacggagggcctgttgatggtgtttaaagacaacattattccctactcgtttaaggtccgctcctacaccaagatagtgaccaacattctcatctacaatggctggtacgcggactccgtgaccaaccggcacgaggagaagttctccgttgacagctacgaaactgaccagatggataccatctaccagtgctacaacgcggtcaagatgacaaaagatgggctgacgcgcgtgtatgtagaccgcgacggagttaacatcaccgtcaacctaaagcccaccgggggcctggccaacggggtgcgccgctacgccagccagacggagctctatgacgcccccgggtggttgatatggacttacagaacaagaactaccgtcaactgcctgataactgacatgatggccaagtccaacagccccttcgacttctttgtgaccaccaccgggcagactgtggaaatgtcccctttctatgacgggaaaaataaggaaaccttccatgagcgggcagactccttccacgtgagaactaactacaagatagtggactacgacaaccgagggacgaacccgcaaggcgaacgccgagccttcctggacaagggcacttacaccctatcttggaagctcgagaacaggacagcctactgcccgcttcaacactggcaaacctttgactcgaccatcgccacagaaacagggaagtcaatacattttgtgactgacgagggcacctctagcttcgtgaccaacacaaccgtgggcatagagctcccggacgccttcaagtgcatcgaagagcaggtgaacaagaccatgcatgagaagtacgaggccgtccaggatcgttacacgaagggccaggaagccattacatattttataacgagcggaggattgttattagcttggctacctctgaccccgcgctcgttggccaccgtcaagaacctgacggagcttaccactccgacttcctcaccccccagcagtccatcgccccccgccccacccgcggcccgcgggagcacctccgccgccgttctgaggcgcggtggcggagggagtggtggcggagggagcggtggcggagggagtgcggggaatgccaccacaccggtgccccccgcggcccccgggaagtccctgggcaccctcaacaatcccgccaccgtccagatccaatttgcctacgattccctgcgccgccagatcaaccgcatgctgggagacctcgcgcgggcctggtgcctggagcagaagaggcagaacatggtgctgagagaactaaccaagattaatcccaccaccgtcatgtccagcatctacggtaaggcggtggcggccaagcgcctgggggatgtcatctcagtctcccagtgcgtgcccgttaaccaggccaccgtcaccctgcgcaagagcatgagggtccctggctccgagaccatgtgctactcgcgccccctggtgtccttcagctttatcaacgacaccaagacctacgagggacagctgggcaccgacaacgagatcttcctcacaaaaaagatgacggaggtgtgccaggcgaccagccagtactacttccagtccggcaacgagatccacgtctacaacgactaccaccactttaaaaccatcgagctggacggcattgccaccctgcagaccttcatctcactaaacacctccctcatcgagaacattgactttgcctccctggagctgtactcacgggacgaacagcgtgcctccaacgtctttgacctggagggcatcttccgggagtacaacttccaggcgcaaaacatcgccggcctgcggaaggatttggacaatgcagtgtcaaacggaagaaatcaattcgtggacggcctgggggaacttatggacagtctgggtagcgtgggtcagtccatcaccaacctagtcagcacggtggggggtttgtttagcagcctggtctctggtttcatctccttcttcaaaaacccctaa

SEQ ID NO: 10 - protein, 743 aa, Epstein-Barr virus
METDTLLLWVLLLWVPGSTGDAAQTPEQPAPPATTVQPTATRQQTSFPFRVCELSSHGDLFRFSSDIQCPSFGTRENHTEGLLMVFKDNIIPYSFKVRSYTKIVTNILIYNGWYADSVTNRHEEKFSVDSYETDQMDTIYQCYNAVKMTKDGLTRVYVDRDGVNITVNLKPTGGLANGVRRYASQTELYDAPGWLIWTYRTRTTVNCLITDMMAKSNSPFDFFVTTTGQTVEMSPFYDGKNKETFHERADSFHVRTNYKIVDYDNRGTNPQGERRAFLDKGTYTLSWKLENRTAYCPLQHWQTFDSTIATETGKSIHFVTDEGTSSFVTNTTVGIELPDAFKCIEEQVNKTMHEKYEAVQDRYTKGQEAITYFITSGGLLLAWLPLTPRSLATVKNLTELTTPTSSPPSSPSPPAPPAARGSTSAAVLRGGGGSGGGGSGGGGSAGNATTPVPPAAPGKSLGTLNNPATVQIQFAYDSLRRQINRMLGDLARAWCLEQKRQNMVLRELTKINPTTVMSSIYGKAVAAKRLGDVISVSQCVPVNQATVTLRKSMRVPGSETMCYSRPLVSFSFINDTKTYEGQLGTDNEIFLTKKMTEVCQATSQYYFQSGNEIHVYNDYHHFKTIELDGIATLQTFISLNTSLIENIDFASLELYSRDEQRASNVFDLEGIFREYNFQAQNIAGLRKDLDNAVSNGRNQFVDGLGELMDSLGSVGQSITNLVSTVGGLFSSLVSGFISFFKNP

SEQ ID NO: 11 - DNA, 2715 bp, Herpes simplex virus 1
atgcgccagggcgcccccgcgcgggggcgccggtggttcgtcgtatgggcgctcttggggttgacgctgggggtcctggtggcgtcggcggctccgagttcccccggcacgcctggggtcgcggccgcgacccaggcggcgaacgggggccctgccactccggcgccgcccgcccctggcgcccccccaacgggggacccgaaaccgaagaagaacagaaaaccgaaacccccaaagccgccgcgccccgccggcgacaacgcgaccgtcgccgcgggccacgccaccctgcgcgagcacctgcgggacatcaaggcggagaacaccgatgcaaacttttacgtgtgcccaccccccacgggcgccacggtggtgcagttcgagcagccgcgccgctgcccgacccggcccgagggtcagaactacacggagggcatcgcggtggtcttcaaggagaacatcgccccgtacaagttcaaggccaccatgtactacaaagacgtcaccgtttcgcaggtgtggttcggccaccgctactcccagtttatggggatctttgaggaccgcgcccccgtccccttcgaggaggtgatcgacaagatcaacgccaagggggtctgtcggtccacggccaagtacgtgcgcaacaacctggagaccaccgcgtttcaccgggacgaccacgagaccgacatggagctgaaaccggccaacgccgcgacccgcacgagccggggctggcacaccaccgacctcaagtacaacccctcgcgggtggaggcgttccaccggtacgggacgacggtaaactgcatcgtcgaggaggtggacgcgcgctcggtgtacccgtacgacgagtttgtgttggcgactggcgactttgtgtacatgtccccgttttacggctaccgggaggggtcgcacaccgaacacaccagctacgccgccgaccgcttcaagcaggtcgacggcttctacgcgcgcgacctcaccaccaaggcccgggccacggcgccgaccacccggaacctgctcacgacccccaagttcaccgtggcctgggactgggtgccaaagcgcccgtcggtctgcaccatgaccaagtggcaggaggtggacgagatgctgcgctccgagtacggcggctccttccgattctcttccgacgccatatccaccaccttcaccaccaacctgaccgagtacccgctctcgcgcgtggacctgggggactgcatcggcaaggacgcccgcgacgccatggaccgcatcttcgcccgcaggtacaacgcgacgcacatcaaggtgggccagccgcagtactacctggccaatgggggctttctgatcgcgtaccagccccttctcagcaacacgctcgcggagctgtacgtgcgggaacacctccgcgagcagagccgcaagcccccaaaccccacgcccccgccgcccggggccagcgccaacgcgtccgtggagcgcatcaagaccacctcctccatcgagttcgccaggctgcagtttacgtacaaccacatacagcgccatgtcaacgatatgttgggccgcgttgccatcgcgtggtgcgagctgcagaatcacgagctgaccctgtggaacgaggcccgcaagctgaaccccaacgccatcgcctcggccaccgtgggccggcgggtgagcgcgcggatgctcggcgacgtgatggccgtctccacgtgcgtgccggtcgccgcggacaacgtgatcgtccaaaactcgatgcgcatcagctcgcggcccggggcctgctacagccgccccctggtcagctttcggtacgaagaccagggcccgttggtcgaggggcagctgggggagaacaacgagctgcggctgacgcgcgatgcgatcgagccgtgcaccgtgggacaccggcgctacttcaccttcggtgggggctacgtgtacttcgaggagtacgcgtactcccaccagctgagccgcgccgacatcaccaccgtcagcaccttcatcgacctcaacatcaccatgctggaggatcacgagtttgtccccctggaggtgtacacccgccacgagatcaaggacagcggcctgctggactacacggaggtccagcgccgcaaccagctgcacgacctgcgcttcgccgacatcgacacggtcatccacgccgacgccaacgccgccatgtttgcgggcctgggcgcgttcttcgaggggatgggcgacctggggcgcgcggtcggcaaggtggtgatgggcatcgtgggcggcgtggtatcggccgtgtcgggcgtgtcctccttcatgtccaacccctttggggcgctggccgtgggtctgttggtcctggccggcctggcggcggccttcttcgcctttcgctacgtcatgcggctgcagagcaaccccatgaaggccctgtacccgctaaccaccaaggagctcaagaaccccaccaacccggacgcgtccggggagggcgaggagggcggcgactttgacgaggccaagctagccgaggcccgggagatgatacggtacatggccctggtgtctgccatggagcgcacggaacacaaggccaagaagaagggcacgagcgcgctgctcagcgccaaggtcaccgacatggtcatgcgcaagcgccgcaacaccaactacacccaagttcccaacaaagacggtgacgccgacgaggacgacctgtga

SEQ ID NO: 12 - protein, 904 aa, Herpes simplex virus 1
MRQGAPARGCRWFVVWALLGLTLGVLVASAAPSSPGTPGVAAATQAANGGPATPAPPALGAAPTGDPKPKKNKKPKNPTPPRPAGDNATVAAGHATLREHLRDIKAESTDANFYVCPPPTGATVVQFEQPRRCPTRPEGQNYTEGIAVVFKENIAPYKFKATMYYKDVTVSQVWFGHRYSQFMGIFEDRAPVPFEEVIDKINAKGVCRSTAKYVRNNLETTAFHRDDHETDMELKPANAATRTSRGWHTTDLKYNPSRVEAFHRYGTTVNCIVEEVDARSVYPYDEFVLATGDFVYMSPFYGYREGSHTEHTSYAADRFKQVDGFYARDLTTKARATAPTTRNLLTTPKFTVAWDWVPKRPSVCTMTKWQEVDEMLRSEYGGSFRFSSDAISTTFTTNLTEYPLSRVDLGDCIGKDARDAMDRIFARRYNATHIKVGQPQYYLANGGFLIAYQPLLSNTLAELYVREHLREQSRKPPNPTPPPPGASANASVERIKTTSSIEFARLQFTYNHIQRHVNDMLGRVAIAWCELQNHELTLWNEARKLNPNAIASATVGRRVSARMLGDVMAVSTCVPVAADNVIVQNSMRISSRPGACYSRPLVSFRYEDQGPLVEGQLGENNELRLTRDAIEPCTVGHRRYFTFGGGYVYFEEYAYSHQLSRADITTVSTFIDLNITMLEDHEFVPLEVYTRHEIKDSGLLDYTEVQRRNQLHDLRFADIDTVIHADANAAMFAGLGAFFEGMGDLGRAVGKVVMGIVGGVVSAVSGVSSFMSNPFGALAVGLLVLAGLAAAFFAFRYVMRLQSNPMKALYPLTTKELKNPTNPDASGEGEEGGDFDEAKLAEAREMIRYMALVSAMEHTEHKAKKKGTSALLSAKVTDMVMRKRRNTNYTQVPNKDGDADEDDL

SEQ ID NO: 13 - DNA, 2751 bp, Herpes simplex virus 2
atgcgcggggggggcttgatttgcgcgctggtcgtgggggcgctggtggccgcggtggcgtcggcggccccggcggccccggcggccccccgcgcctcgggcggcgtggccgcgaccgtcgcggcgaacgggggtcccgcctcccggccgccccccgtcccgagccccgcgaccaccaaggcccggaagcggaaaaccaaaaagccgcccaagcggcccgaggcgaccccgccccccgacgccaacgcgaccgtcgccgccggccacgccacgctgcgcgcgcacctgcgggaaatcaaggtcgagaacgccgatgcccagttttacgtgtgcccgcccccgacgggcgccacggtggtgcagtttgagcagccgcgccgctgcccgacgcgcccggaggggcagaactacacggagggcatcgcggtggtcttcaaggagaacatcgccccgtacaaattcaaggccaccatgtactacaaagacgtgaccgtgtcgcaggtgtggttcggccaccgctactcccagtttatggggatattcgaggaccgcgcccccgttcccttcgaggaggtgatcgacaagattaacaccaagggggtctgccgctccacggccaagtacgtgcggaacaacatggagaccaccgcgtttcaccgggacgaccacgagaccgacatggagctcaagccggcgaaggtcgccacgcgcacgagccgggggtggcacaccaccgacctcaagtacaacccctcgcgggtggaggcgttccatcggtacggcacgacggtcaactgcatcgtcgaggaggtggacgcgcggtcggtgtacccgtacgatgagtttgtgctggcgacgggcgactttgtgtacatgtccccgttttacggctaccgggaggggtcgcacaccgagcacaccagctacgccgccgaccgcttcaagcaggtcgacggcttctacgcgcgcgacctcaccacgaaggcccgggccacgtcgccgacgacccgcaacttgctgacgacccccaagtttaccgtggcctgggactgggtgccgaagcgaccggcggtctgcaccatgaccaagtggcaggaggtggacgagatgctccgcgccgagtacggcggctccttccgcttctcctccgacgccatctcgaccaccttcaccaccaacctgaccgagtactcgctctcgcgcgtcgacctgggcgactgcatcggccgggatgcccgcgaggccatcgaccgcatgtttgcgcgcaagtacaacgccacgcacatcaaggtgggccagccgcagtactacctggccacggggggcttcctcatcgcgtaccagcccctcctcagcaacacgctcgccgagctgtacgtgcgggagtacatgcgggagcaggaccgcaagccccggaatgccacgcccgcgccactgcgggaggcgcccagcgccaacgcgtccgtggagcgcatcaagaccacctcctcgatcgagttcgcccggctgcagtttacgtataaccacatacagcgccacgtgaatgacatgctggggcgcatcgccgtcgcgtggtgcgagctgcagaaccacgagctgactctctggaacgaggcccgcaagctcaaccccaacgccatcgcctccgccaccgtcggccggcgggtgagcgcgcgcatgctcggagacgtcatggccgtctccacgtgcgtgcccgtcgccccggacaacgtgatcgtgcagaactcgatgcgcgtcagctcgcggccggggacgtgctacagccgccccctggtcagctttcggtacgaagaccagggcccgctgatcgaggggcagctgggcgagaacaacgagctgcgcctcacccgcgacgcgctcgagccgtgcaccgtgggccaccggcgctacttcatcttcggcgggggctacgtgtacttcgaggagtacgcgtactctcaccagctgagtcgcgccgacgtcaccaccgtcagcaccttcatcgacctgaacatcaccatgctggaggaccacgagtttgtgcccctggaggtctacacgcgccacgagatcaaggacagcggcctgctggactacacggaggtccagcgccgcaaccagctgcacgacctgcgctttgccgacatcgacacggtcatccgcgccgacgccaacgccgccatgttcgcggggctgtgcgcgttcttcgaggggatgggggacttggggcgcgcggtcggcaaggtagtcatgggagtagtggggggcgtggtgtcggccgtctcgggcgtgtcctcctttatgtccaaccccttcggggcgcttgccgtggggctgctggtcctggccggcctggtcgcggccttcttcgccttccgctacgtcctgcaactgcaacgcaatcccatgaaggccctgtatccgctcaccaccaaggaactcaagacttccgaccccgggggcgtgggcggggagggggaggaaggcgcggaggggggcgggtttgacgaggccaagttggccgaggcccgagaaatgatccgatatatggctttggtgtcggccatggagcgcacggaacacaaggccagaaagaagggcacgagcgccctgctcagctccaaggtcaccaacatggttctgcgcaagcgcaacaaagccaggtactctccgctccacaacgaggacgaggccggagacgaagacgagctctaagggaggggaggggagctgggcttgtgtataaataaa

SEQ ID NO: 14 - protein, 904 aa, Herpes simplex virus 2
MRGGGLICALVVGALVAAVASAAPAAPAAPRASGGVAATVAANGGPASRPPPVPSPATTKARKRKTKKPPKRPEATPPPDANATVAAGHATLRAHLREIKVENADAQFYVCPPPTGATVVQFEQPRRCPTRPEGQNYTEGIAVVFKENIAPYKFKATMYYKDVTVSQVWFGHRYSQFMGIFEDRAPVPFEEVIDKINTKGVCRSTAKYVRNNMETTAFHRDDHETDMELKPAKVATRTSRGWHTTDLKYNPSRVEAFHRYGTTVNCIVEEVDARSVYPYDEFVLATGDFVYMSPFYGYREGSHTEHTSYAADRFKQVDGFYARDLTTKARATSPTTRNLLTTPKFTVAWDWVPKRPAVCTMTKWQEVDEMLRAEYGGSFRFSSDAISTTFTTNLTEYSLSRVDLGDCIGRDAREAIDRMFARKYNATHIKVGQPQYYLATGGFLIAYQPLLSNTLAELYVREYMREQDRKPRNATPAPLREAPSANASVERIKTTSSIEFARLQFTYNHIQRHVNDMLGRIAVAWCELQNHELTLWNEARKLNPNAIASATVGRRVSARMLGDVMAVSTCVPVAPDNVIVQNSMRVSSRPGTCYSRPLVSFRYEDQGPLIEGQLGENNELRLTRDALEPCTVGHRRYFIFGGGYVYFEEYAYSHQLSRADVTTVSTFIDLNITMLEDHEFVPLEVYTRHEIKDSGLLDYTEVQRRNQLHDLRFADIDTVIRADANAAMFAGLCAFFEGMGDLGRAVGKVVMGVVGGVVSAVSGVSSFMSNPFGALAVGLLVLAGLVAAFFAFRYVLQLQRNPMKALYPLTTKELKTSDPGGVGGEGEEGAEGGGFDEAKLAEAREMIRYMALVSAMERTEHKARKKGTSALLSSKVTNMVLRKRNKARYSPLHNEDEAGDEDEL

SEQ ID NO: 15 - DNA, 2796 bp, Varicella zoster virus
atgtccccttgtggctattattcaaagtggagaaacagggatcgaccagaataccgtcgtaatctacgattcagacgttttttctcttctatacaccctaatgcagcggctggctccggattcaacggacccggcgttttcataacctccgttacgggggtgtggttatgctttttatgcatattttctatgtttgttacggcggttgtgtcggtctctccaagctcgttttatgagagtttacaagtagagcccacacaatcagaagatataacccggtctgctcatctgggcgatggtgatgaaatcagagaagctatacacaagtcccaggacgccgaaacaaaacccacgttttacgtctgcccaccgccaacaggctccacaatcgtacgattagaaccaactcggacatgtccggattatcaccttggtaaaaactttacagagggtattgctgttgtttataaagaaaacattgcagcgtacaagtttaaggcgacggtatattacaaagatgttatcgttagcacggcgtgggccggaagttcttatacgcaaattactaatagatatgcggatagggtaccaattcccgtttcagagatcacggacaccattgataagtttggcaagtgttcttctaaagcaacgtacgtacgaaataaccacaaagttgaagcctttaatgaggataaaaatccacaggatatgcctctaatcgcatcaaaatataattctgtgggatccaaagcatggcatactaccaatgacacgtacatggttgccggaacccccggaacatataggacgggcacgtcggtgaattgcatcattgaggaagttgaagccagatcaatattcccttatgatagttttggactttccacgggagatataatatacatgtccccgttttttggcctacgggatggtgcatacagagaacattccaattatgcaatggatcgttttcaccagtttgagggttatagacaaagggatcttgacactagagcattactggaacctgcagcgcggaactttttagtcacgcctcatttaacggttggttggaactggaagccaaaacgaacggaagtttgttcgcttgtcaagtggcgtgaggttgaagacgtagttcgcgatgagtatgcacacaattttcgctttacaatgaaaacactttctaccacgtttataagtgaaacaaacgagtttaatcttaaccaaatccatctcagtcaatgtgtaaaggaggaagcccgggctattattaaccggatctatacaaccagatacaactcatctcatgttagaaccggggatatccagacctaccttgccagaggggggtttgttgtggtgtttcaacccctgctgagcaattccctcgcccgtctctatctccaagaattggtccgtgaaaacactaatcattcaccacaaaaacacccgactcgaaataccagatcccgacgaagcgtgccagttgagttgcgtgccaatagaacaataacaaccacctcatcggtggaatttgctatgctccagtttacatatgaccacattcaagagcatgttaatgaaatgttggcacgtatctcctcgtcgtggtgccagctacaaaatcgcgaacgcgccctttggagcggactatttccaattaacccaagtgctttagcgagcaccattttggatcaacgtgttaaagctcgtattctcggcgacgttatctccgtttctaattgtccagaactgggatcagatacacgcattatacttcaaaactctatgagggtatctggtagtactacgcgttgttatagccgtcctttaatttcaatagttagtttaaatgggtccgggacggtggagggccagcttggaacagataacgagttaattatgtccagagatctgttagaaccatgcgtggctaatcacaagcgatattttctatttgggcatcactacgtatattatgaggattatcgttacgtccgtgaaatcgcagtccatgatgtgggaatgattagcacttacgtagatttaaacttaacacttcttaaagatagagagtttatgccgctgcaagtatatacaagagacgagctgcgggatacaggattactagactacagtgaaattcaacgccgaaatcaaatgcattcgctgcgtttttatgacatagacaaggttgtgcaatatgatagcggaacggccattatgcagggcatggctcagtttttccagggacttgggaccgcgggccaggccgttggacatgtggttcttggggccacgggagcgctgctttccaccgtacacggatttaccacgtttttatctaacccatttggggcattggccgtgggattattggttttggcgggactggtagcggccttttttgcgtaccggtacgtgcttaaacttaaaacaagcccgatgaaggcattatatccactcacaaccaaggggttaaaacagttaccggaaggaatggatccctttgccgagaaacccaacgctactgataccccaatagaagaaattggcgactcacaaaacactgaaccgtcggtaaatagcgggtttgatcccgataaatttcgagaagcccaggaaatgattaaatatatgacgttagtatctgcggctgagcgccaagaatctaaagcccgcaaaaaaaataagactagcgcccttttaacttcacgtcttaccggccttgctttacgaaatcgccgaggatactcccgtgttcgcaccgagaatgtaacgggggtgtaa

SEQ ID NO: 16 - protein, 931 aa, Varicella zoster virus
MSPCGYYSKWRNRDRPEYRRNLRFRRFFSSIHPNAAAGSGFNGPGVFITSVTGVWLCFLCIFSMFVTAVVSVSPSSFYESLQVEPTQSEDITRSAHLGDGDEIREAIHKSQDAETKPTFYVCPPPTGSTIVRLEPTRTCPDYHLGKNFTEGIAVVYKENIAAYKFKATVYYKDVIVSTAWAGSSYTQITNRYADRVPIPVSEITDTIDKFGKCSSKATYVRNNHKVEAFNEDKNPQDMPLIASKYNSVGSKAWHTTNDTYMVAGTPGTYRTGTSVNCIIEEVEARSIFPYDSFGLSTGDIIYMSPFFGLRDGAYREHSNYAMDRFHQFEGYRQRDLDTRALLEPAARNFLVTPHLTVGWNWKPKRTEVCSLVKWREVEDVVRDEYAHNFRFTMKTLSTTFISETNEFNLNQIHLSQCVKEEARAIINRIYTTRYNSSHVRTGDIQTYLARGGFVVVFQPLLSNSLARLYLQELVRENTNHSPQKHPTRNTRSRRSVPVELRANRTITTTSSVEFAMLQFTYDHIQEHVNEMLARISSSWCQLQNRERALWSGLFPINPSALASTILDQRVKARILGDVISVSNCPELGSDTRIILQNSMRVSGSTTRCYSRPLISIVSLNGSGTVEGQLGTDNELIMSRDLLEPCVANHKRYFLFGHHYVYYEDYRYVREIAVHDVGMISTYVDLNLTLLKDREFMPLQVYTRDELRDTGLLDYSEIQRRNQMHSLRFYDIDKVVQYDSGTAIMQGMAQFFQGLGTAGQAVGHVVLGATGALLSTVHGFTTFLSNPFGALAVGLLVLAGLVAAFFAYRYVLKLKTSPMKALYPLTTKGLKQLPEGMDPFAEKPNATDTPIEEIGDSQNTEPSVNSGFDPDKFREAQEMIKYMTLVSAAERQESKARKKNKTSALLTSRLTGLALRNRRGYSRVRTENVTGV

SEQ ID NO: 17 - DNA, 2229 bp, Human cytomegalovirus
atgcggccaggcctcccctcctacctcatcatcctcgccgtctgtctcttcagccacctactttcgtcacgatatggcgcagaagccgtatccgaaccgctggacaaagcgtttcacctactgctcaacacctacgggagacccatccgcttcctgcgtgaaaataccacccagtgtacctacaacagcagcctccgtaacagcacggtcgtcagggaaaacgccatcagtttcaactttttccaaagctataatcaatactatgtattccatatgcctcgatgtctttttgcgggtcctctggcggagcagtttctgaaccaggtagatctgaccgaaaccctggaaagataccaacagagacttaacacttacgcgctggtatccaaagacctggccagctaccgatctttttcgcagcagctaaaggcacaagacagcctaggtgaacagcccaccactgtgccaccgcccattgacctgtcaatacctcacgtttggatgccaccgcaaaccactccacacggctggacagaatcacataccacctcaggactacaccgaccacactttaaccagacctgtatcctctttgatggacacgatctactattcagcaccgtcacaccttgtttgcaccaaggcttttacctcatcgacgaactacgttacgttaaaataacactgaccgaggacttcttcgtagttacggtgtccatagacgacgacacacccatgctgcttatcttcggccatcttccacgcgtacttttcaaagcgccctatcaacgcgacaactttatactacgacaaactgaaaaacacgagctcctggtgctagttaagaaagatcaactgaaccgtcactcttatctcaaagacccggactttcttgacgccgcacttgacttcaactacctagacctcagcgcactactacgtaacagctttcaccgttacgccgtggatgtactcaagagcggtcgatgtcagatgctggaccgccgcacggtagaaatggccttcgcctacgcattagcactgttcgcagcagcccgacaagaagaggccggcgcccaagtctccgtcccacgggccctagaccgccaggccgcactcttacaaatacaagaatttatgatcacctgcctctcacaaacaccaccacgcaccacgttgctgctgtatcccacggccgtggacctggccaaacgagccctttggacaccgaatcagatcaccgacatcaccagcctcgtacgcctggtctacatactctctaaacagaatcagcaacatctcatcccccaatgggcactacgacagatcgccgactttgccctaaaactacacaaaacgcacctggcctcttttctttcagccttcgcacgccaagaactctacctcatgggcagcctcgtccactccatgctggtacatacgacggagagacgcgaaatcttcatcgtagaaacgggcctctgttcattggccgagctatcacactttacgcagttgttagctcatccacaccacgaatacctcagcgacctgtacacaccctgttccagtagcgggcgacgcgatcactcgctcgaacgcctcacgcgtctcttccccgatgccaccgtccccgctaccgttcccgccgccctctccatcctatctaccatgcaaccaagcacgctggaaaccttccccgacctgttttgcttgccgctcggcgaatccttctccgcgctgaccgtctccgaacacgtcagttatatcgtaacaaaccagtacctgatcaaaggtatctcctaccctgtctccaccaccgtcgtaggccagagcctcatcatcacccagacggacagtcaaactaaatgcgaactgacgcgcaacatgcataccacacacagcatcacagtggcgctcaacatttcgctagaaaactgcgccttttgccaaagcgccctgctagaatacgacgacacgcaaggcgtcatcaacatcatgtacatgcacgactcggacgacgtccttttcgccctggatccctacaacgaagtggtggtctcatctccgcgaactcactacctcatgcttttgaaaaacggtacggtactagaagtaactgacgtcgtcgtggacgccaccgacagtcgtctcctcatgatgtccgtctacgcgctatcggccatcatcggcatctatctgctctaccgcatgctcaagacatgctga

SEQ ID NO: 18 - protein, 742 aa, Human cytomegalovirus
MRPGLPSYLIVLAVCLLSHLLSSRYGAEAISEPLDKAFHLLLNTYGRPIRFLRENTTQCTYNSSLRNSTVVRENAISFNFFQSYNQYYVFHMPRCLFAGPLAEQFLNQVDLTETLERYQQRLNTYALVSKDLASYRSFSQQLKAQDSLGEQPTTVPPPIDLSIPHVWMPPQTTPHGWTESHTTSGLHRPHFNQTCILFDGHDLLFSTVTPCLHQGFYLIDELRYVKITLTEDFFVVTVSIDDDTPMLLIFGHLPRVLFKAPYQRDNFILRQTEKHELLVLVKKDQLNRHSYLKDPDFLDAALDFNYLDLSALLRNSFHRYAVDVLKSGRCQMLDRRTVEMAFAYALALFAAARQEEAGAQVSVPRALDRQAALLQIQEFMITCLSQTPPRTTLLLYPTAVDLAKRALWTPNQITDITSLVRLVYILSKQNQQHLIPQWALRQIADFALKLHKTHLASFLSAFARQELYLMGSLVHSMLVHTTERREIFIVETGLCSLAELSHFTQLLAHPHHEYLSDLYTPCSSSGRRDHSLERLTRLFPDATVPTTVPAALSILSTMQPSTLETFPDLFCLPLGESFSALTVSEHVSYVVTNQYLIKGISYPVSTTVVGQSLIITQTDSQTKCELTRNMHTTHSITAALNISLENCAFCQSALLEYDDTQGVINIMYMHDSDDVLFALDPYNEVVVSSPRTHYLMLLKNGTVLEVTDVVVDATDSRLLMMSVYALSAIIGIYLLYRMLKTC

SEQ ID NO: 19 - protein, 5 aa, Human cytomegalovirus
RTKRS

SEQ ID NO: 20 - protein, 5 aa, Epstein-Barr virus
RRRRD

SEQ ID NO: 21 - DNA, 2229 bp, Human herpesvirus
tcagcatgtcttgagcatgcggtagagcagatagatgccgatgatggccgatagcgcgtagacggacatcatgaggagacgactgtcggtggcgtccacgacgacgtcagttacttctagtaccgtaccgtttttcaaaagcatgaggtagtgagttcgcggagatgagaccaccacttcgttgtagggatccagggcgaaaaggacgtcgtccgagtcgtgcatgtacatgatgttgatgacgccttgcgtgtcgtcgtattctagcagggcgctttggcaaaaggcgcagttttctagcgaaatgttgagcgccactgtgatgctgtgtgtggtatgcatgttgcgcgtcagttcgcatttagtttgactgtccgtctgggtgatgatgaggctctggcctacgacggtggtggagacagggtaggagatacctttgatcaggtactggtttgttacgatataactgacgtgttcggagacggtcagcgcggagaaggattcgccgagcggcaagcaaaacaggtcggggaaggtttccagcgtgcttggttgcatggtagataggatggagagggcggcgggaacggtagcggggacggtggcatcggggaagagacgcgtgaggcgttcgagcgagtgatcgcgtcgcccgctactggaacagggtgtgtacaggtcgctgaggtattcgtggtgtggatgagctaacaactgcgtaaagtgtgatagctcggccaatgaacagaggcccgtttctacgatgaagatttcgcgtctctccgtcgtatgtaccagcatggagtggacgaggctgcccatgaggtagagttcttggcgtgcgaaggctgaaagaaaagaggccaggtgcgttttgtgtagttttagggcaaagtcggcgatctgtcgtagtgcccattgggggatgagatgttgctgattctgtttagagagtatgtagaccaggcgtacgaggctggtgatgtcggtgatctgattcggtgtccaaagggctcgtttggccaggtccacggccgtgggatacagcagcaacgtggtgcgtggtggtgtttgtgagaggcaggtgatcataaattcttgtatttgtaagagtgcggcctggcggtctagggcccgtgggacggagacttgggcgccggcctcttcttgtcgggctgctgcgaacagtgctaatgcgtaggcgaaggccatttctaccgtgcggcggtccagcatctgacatcgaccgctcttgagtacatccacggcgtaacggtgaaagctgttacgtagtagtgcgctgaggtctaggtagttgaagtcaagtgcggcgtcaagaaagtccgggtctttgagataagagtgacggttcagttgatctttcttaactagcaccaggagctcgtgtttttcagtttgtcgtagtataaagttgtcgcgttgatagggcgctttgaaaagtacgcgtggaagatggccgaagataagcagcatgggtgtgtcgtcgtctatggacaccgtaactacgaagaagtcctcggtcagtgttattttaacgtaacgtagttcgtcgatgaggtaaaagccttggtgcaaacaaggtgtgacggtgctgaatagtagatcgtgtccatcaaagaggatacaggtctggttaaagtgtggtcggtgtagtcctgaggtggtatgtgattctgtccagccgtgtggagtggtttgcggtggcatccaaacgtgaggtattgacaggtcaatgggcggtggcacagtggtgggctgttcacctaggctgtcttgtgcctttagctgctgcgaaaaagatcggtagctggccaggtctttggataccagcgcgtaagtgttaagtctctgttggtatctttccagggtttcggtcagatctacctggttcagaaactgctccgccagaggacccgcaaaaagacatcgaggcatatggaatacatagtattgattatagctttggaaaaagttgaaactgatggcgttttccctgacgaccgtgctgttacggaggctgctgttgtaggtacactgggtggtattttcacgcaggaagcggatgggtctcccgtaggtgttgagcagtaggtgaaacgctttgtccagcggttcggatacggcttctgcgccatatcgtgacgaaagtaggtggctgaagagacagacggcgaggatgatgaggtaggaggggaggcctggccgcat

SEQ ID NO: 22 - DNA, 837 bp, Human herpesvirus
ttagcgagcatccactgcttgagggccatagcgcgagtgagccggcaggttgacgcgcgtctgcttcagctcgggcggcagtccggcgtagtatttatctaggtggcgtagcagcggcgggtccagctggtgacgcaggcagaattccttcactgcgttgtacaggccgtaaaagagcgtgatgccctcgggcgcggcagcggtgctcacgggcagacgcacggcgcggttggtacgcgtggcttcgttgcgtatggccaccaccacgttaaagagagacggtggcaccagctcgaagcctaacacgtgttccgtgaagatgctgcgcccgtatgacagtcgcgtgaggtcgtagccgcggcacaggtcgtccacgcacgtgtacacggccggcgagccatcgccgcactcgctgtagccgcgcatcaccgtcatccagcgcggcgctgtgtccgagctcaacagcgtcagcagggcccgcaattgatccggattgttgtacagcagggccagagtgtccaggaaagcctcgtccaacagcacggagttggcggcctccggcgtaacgggacggtaacggataagttgcgatagcgggccatcgcgcccggtaacattcaccaacgggcgcagccaactttcatacttgtcaccctcaaacacctcacccaacaagcatcggcgcgttagttcggggcactccgcggggactttctcggcggcggtaggagcgacgctgacggcggctgaggaaacaatgggcagcagaaggcaacaccacagcagtatcaccggtccaggtgagaaagagaagccgcaatccgggcggcggcacat

SEQ ID NO: 23 - DNA, 837 bp, Human cytomegalovirus
atgtgccgccgcccggattgcggcttctctttctcacctggaccggtgatactgctgtggtgttgccttctgctgcccattgtttcctcagccgccgtcagcgtcgctcctaccgccgccgagaaagtccccgcggagtgccccgaactaacgcgccgatgcttgttgggtgaggtgtttgagggtgacaagtatgaaagttggctgcgcccgttggtgaatgttaccgggcgcgatggcccgctatcgcaacttatccgttaccgtcccgttacgccggaggccgccaactccgtgctgttggacgaggctttcctggacactctggccctgctgtacaacaatccggatcaattgcgggccctgctgacgctgttgagctcggacacagcgccgcgctggatgacggtgatgcgcggctacagcgagtgcggcgatggctcgccggccgtgtacacgtgcgtggacgacctgtgccgcggctacgacctcacgcgactgtcatacgggcgcagcatcttcacggaacacgtgttaggcttcgagctggtgccaccgtctctctttaacgtggtggtggccatacgcaacgaagccacgcgtaccaaccgcgccgtgcgtctgcccgtgagcaccgctgccgcgcccgagggcatcacgctcttttacggcctgtacaacgcagtgaaggaattctgcctgcgtcaccagctggacccgccgctgctacgccacctagataaatactacgccggactgccgcccgagctgaagcagacgcgcgtcaacctgccggctcactcgcgctatggccctcaagcagtggatgctcgctaa

SEQ ID NO: 24 - protein, 278 aa, Human cytomegalovirus
MCRRPDCGFSFSPGPVALLWCCLLLPIVSSATVSVAPTVAEKVPAECPELTRRCLLGEVFQGDKYESWLRPLVNVTRRDGPLSQLIRYRPVTPEAANSVLLDDAFLDTLALLYNNPDQLRALLTLLSSDTAPRWMTVMRGYSECGDGSPAVYTCVDDLCRGYDLTRLSYGRSIFTEHVLGFELVPPSLFNVVVAIRNEATRTNRAVRLPVSTAAAPEGITLFYGLYNAVKEFCLRHQLDPPLLRHLDKYYAGLPPELKQTRVNLPAHSRYGPQAVDAR

SEQ ID NO: 25 - protein, 984 aa, Human cytomegalovirus
METDTLLLWVLLLWVPGSTGDATVSVAPTVAEKVPAECPELTRRCLLGEVFQGDKYESWLRPLVNVTRRDGPLSQLIRYRPVTPEAANSVLLDDAFLDTLALLYNNPDQLRALLTLLSSDTAPRWMTVMRGYSECGDGSPAVYTCVDDLCRGYDLTRLSYGRSIFTEHVLGFELVPPSLFNVVVAIRNEATRTNRAVRLPVSTAAAPEGITLFYGLYNAVKEFCLRHQLDPPLLRHLDKYYAGLPPELKQTRVNLPAHSRYGPQAVDARGGGGSGGGGSGGGGSYGAEAISEPLDKAFHLLLNTYGRPIRFLRENTTQCTYNSSLRNSTVVRENAISFNFFQSYNQYYVFHMPRCLFAGPLAEQFLNQVDLTETLERYQQRLNTYALVSKDLASYRSFSQQLKAQDSLGEQPTTVPPPIDLSIPHVWMPPQTTPHGWTESHTTSGLHRPHFNQTCILFDGHDLLFSTVTPCLHQGFYLIDELRYVKITLTEDFFVVTVSIDDDTPMLLIFGHLPRVLFKAPYQRDNFILRQTEKHELLVLVKKDQLNRHSYLKDPDFLDAALDFNYLDLSALLRNSFHRYAVDVLKSGRCQMLDRRTVEMAFAYALALFAAARQEEAGAQVSVPRALDRQAALLQIQEFMITCLSQTPPRTTLLLYPTAVDLAKRALWTPNQITDITSLVRLVYILSKQNQQHLIPQWALRQIADFALKLHKTHLASFLSAFARQELYLMGSLVHSMLVHTTERREIFIVETGLCSLAELSHFTQLLAHPHHEYLSDLYTPCSSSGRRDHSLERLTRLFPDATVPTTVPAALSILSTMQPSTLETFPDLFCLPLGESFSALTVSEHVSYVVTNQYLIKGISYPVSTTVVGQSLIITQTDSQTKCELTRNMHTTHSITAALNISLENCAFCQSALLEYDDTQGVINIMYMHDSDDVLFALDPYNEVVVSSPRTHYLMLLKNGTVLEVTDVVVDATDSRLHHHHHH

SEQ ID NO: 26 - protein, 6 aa, Artificial Sequence
  Description of Artificial Sequence: Synthetic 6xHis tag
HHHHHH